European Patent Specification EP 3 831 358 B1, published March 12, 2025. Title: Peptides and compositions for use in cosmetics and medicine. Applicant: Lipotrue S.L. The sequence listing filed with the application follows.

SEQUENCE LISTING (4 sequences)

SEQ ID NO: 1 - protein, 6 aa, Artificial Sequence
  Artificially synthesized sequence
RRQMRE

SEQ ID NO: 2 - protein, 6 aa, Artificial Sequence
  Artificially synthesized sequence
MRREQR

SEQ ID NO: 3 - protein, 6 aa, Artificial Sequence
  Artificially synthesized sequence
REQMRR

SEQ ID NO: 4 - protein, 6 aa, Artificial Sequence
  Artificially synthesized sequence
RRQMEE